European Patent Application EP 4 768 505 A1, published July 1, 2026. Title: 一种靶向CD79B的单域抗体和嵌合抗原受体及其应用. Applicant: 深圳市济因生物科技有限公司. Application WO. The sequence listing filed with the application follows.

SEQUENCE LISTING (38 sequences)

SEQ ID NO: 1 - protein, 124 aa, synthetic construct
DVQLQESGGGLVQPGGSLRLSCAASGFAFSLYAMSWARQAPGKGLEWVSDIYGDDDSRRNYADSVKGRFTISRDNAKNTVYLQMTNLQPEDTALYYCGKGRDGTRWSAREYEYRGQGTQVTVSS

SEQ ID NO: 2 - protein, 25 aa, synthetic construct
DVQLQESGGGLVQPGGSLRLSCAAS

SEQ ID NO: 3 - protein, 10 aa, synthetic construct
GFAFSLYAMS

SEQ ID NO: 4 - protein, 14 aa, synthetic construct
WARQAPGKGLEWVS

SEQ ID NO: 5 - protein, 11 aa, synthetic construct
DIYGDDDSRRN

SEQ ID NO: 6 - protein, 38 aa, synthetic construct
YADSVKGRFTISRDNAKNTVYLQMTNLQPEDTALYYCG

SEQ ID NO: 7 - protein, 15 aa, synthetic construct
KGRDGTRWSAREYEY

SEQ ID NO: 8 - protein, 11 aa, synthetic construct
RGQGTQVTVSS

SEQ ID NO: 9 - protein, 116 aa, synthetic construct
DVQLQESGGGLVQPGGSLSLSCAASISSSSIWVRAWHRQAPGKQRELVAAINNDGQTMYADSVKGRFTISRDNAKTTVSLQMNSLKPEDTAVYYCNVVTPKGHQYWGQGTQVTVSS

SEQ ID NO: 10 - protein, 25 aa, synthetic construct
DVQLQESGGGLVQPGGSLSLSCAAS

SEQ ID NO: 11 - protein, 10 aa, synthetic construct
ISSSSIWVRA

SEQ ID NO: 12 - protein, 14 aa, synthetic construct
WHRQAPGKQRELVA

SEQ ID NO: 13 - protein, 9 aa, synthetic construct
AINNDGQTM

SEQ ID NO: 14 - protein, 38 aa, synthetic construct
YADSVKGRFTISRDNAKTTVSLQMNSLKPEDTAVYYCN

SEQ ID NO: 15 - protein, 9 aa, synthetic construct
VVTPKGHQY

SEQ ID NO: 16 - protein, 11 aa, synthetic construct
WGQGTQVTVSS

SEQ ID NO: 17 - protein, 116 aa, synthetic construct
DVQLQESGGGLMQPGGSLSLTCTASISSLSIWVRAWHRQAPGKQRELVAAINSDGQTMYADSVKGRFTISRDSAKTTVSLQMDSLKPEDTAVYYCNVVTPKGQQYWGQGTQVTVSS

SEQ ID NO: 18 - protein, 25 aa, synthetic construct
DVQLQESGGGLMQPGGSLSLTCTAS

SEQ ID NO: 19 - protein, 10 aa, synthetic construct
ISSLSIWVRA

SEQ ID NO: 20 - protein, 9 aa, synthetic construct
AINSDGQTM

SEQ ID NO: 21 - protein, 38 aa, synthetic construct
YADSVKGRFTISRDSAKTTVSLQMDSLKPEDTAVYYCN

SEQ ID NO: 22 - protein, 9 aa, synthetic construct
VVTPKGQQY

SEQ ID NO: 23 - protein, 116 aa, synthetic construct
DVQLQESGGGLVQPGGSLSLSCAASMSSPSLWVRAWHRQAPGKQRELVAAINSDGQTMYADSVKGRFTISRDNAKTLVSLQMDSLKPEDTAVYYCNVVTPRGQQYWGQGTQVTVSS

SEQ ID NO: 24 - protein, 10 aa, synthetic construct
MSSPSLWVRA

SEQ ID NO: 25 - protein, 38 aa, synthetic construct
YADSVKGRFTISRDNAKTLVSLQMDSLKPEDTAVYYCN

SEQ ID NO: 26 - protein, 9 aa, synthetic construct
VVTPRGQQY

SEQ ID NO: 27 - protein, 116 aa, synthetic construct
DVQLQESGGGLVQPGGSLSLTCTASISSLTIWVRAWHRQAPGKQRELVAAINSDGQTMYADSVKGRFTISRDNAKTTVSLQMDSLKPEDTAVYYCNVVTPNGQQYWGQGTQVTVSS

SEQ ID NO: 28 - skipped

SEQ ID NO: 29 - protein, 10 aa, synthetic construct
ISSLTIWVRA

SEQ ID NO: 30 - protein, 38 aa, synthetic construct
YADSVKGRFTISRDNAKTTVSLQMDSLKPEDTAVYYCN

SEQ ID NO: 31 - protein, 9 aa, synthetic construct
VVTPNGQQY

SEQ ID NO: 32 - protein, 21 aa, Homo sapiens
MALPVTALLLPLALLLHAARP

SEQ ID NO: 33 - protein, 45 aa, Homo sapiens
TTTPAPRPPTPAPTIASQPLSLRPEACRPAAGGAVHTRGLDFACD

SEQ ID NO: 34 - protein, 24 aa, Homo sapiens
IYIWAPLAGTCGVLLLSLVITLYC

SEQ ID NO: 35 - protein, 42 aa, Homo sapiens
KRGRKKLLYIFKQPFMRPVQTTQEEDGCSCRFPEEEEGGCEL

SEQ ID NO: 36 - protein, 112 aa, Homo sapiens
RVKFSRSADAPAYQQGQNQLYNELNLGRREEYDVLDKRRGRDPEMGGKPRRKNPQEGLYNELQKDKMAEAYSEIGMKGERRRGKGHDGLYQGLSTATKDTYDALHMQALPPR

SEQ ID NO: 37 - protein, 22 aa, synthetic construct
VKQTLNFDLLKLAGDVESNPGP

SEQ ID NO: 38 - protein, 239 aa, Aequorea victoria
MVSKGEELFTGVVPILVELDGDVNGHKFSVSGEGEGDATYGKLTLKFICTTGKLPVPWPTLVTTLTYGVQCFSRYPDHMKQHDFFKSAMPEGYVQERTIFFKDDGNYKTRAEVKFEGDTLVNRIELKGIDFKEDGNILGHKLEYNYNSHNVYIMADKQKNGIKVNFKIRHNIEDGSVQLADHYQQNTPIGDGPVLLPDNHYLSTQSALSKDPNEKRDHMVLLEFVTAAGITLGMDELYK